European Patent Specification EP 3 599 842 B1, published August 7, 2024. Title: A GENETICALLY MODIFIED MOUSE EXPRESSING HUMAN APOE4 AND MOUSE Trem2 p.R47H. Applicant: The Jackson Laboratory. The sequence listing filed with the application follows.

SEQUENCE LISTING (17 sequences)

SEQ ID NO: 1 - protein, 317 aa, Homo sapiens [sequence omitted]

SEQ ID NO: 2 - DNA, 2792 bp, Homo sapiens
actggccaatcacaggcaggaagatgaaggttctgtgggctgcgttgctggtcacattcctggcaggtatgggggcggggcttgctcggttccccccgctcctccccctctcatcctcacctcaacctcctggccccattcaggcagaccctgggccccctcttctgaggcttctgtgctgcttcctggctctgaacagcgatttgacgctctctgggcctcggtttcccccatccttgagataggagttagaagttgttttgttgttgttgtttgttgttgttgttttgtttttttgagatgaagtctcgctctgtcgcccaggctggagtgcagtggcgggatctcggctcactgcaagctccgcctcccaggtccacgccattctcctgcctcagcctcccaagtagctgggactacaggcacatgccaccacacccgactaacttttttgtattttcagtagagacggggtttcaccatgttggccaggctggtctggaactcctgacctcaggtgatctgcccgtttcgatctcccaaagtgctgggattacaggcgtgagccaccgcacctggctgggagttagaggtttctaatgcattgcaggcagatagtgaataccagacacggggcagctgtgatctttattctccatcacccccacacagccctgcctggggcacacaaggacactcaatacatgcttttccgctgggcgcggtggctcacccctgtaatcccagcactttgggaggccaaggtgggaggatcacttgagcccaggagttcaacaccagcctgggcaacatagtgagaccctgtctctactaaaaatacaaaaattagccaggcatggtgccacacacctgtgctctcagctactcaggaggctgaggcaggaggatcgcttgagcccagaaggtcaaggttgcagtgaaccatgttcaggccgctgcactccagcctgggtgacagagcaagaccctgtttataaatacataatgctttccaagtgattaaaccgactcccccctcaccctgcccaccatggctccaaagaagcatttgtggagcaccttctgtgtgcccctaggtactagatgcctggacggggtcagaaggaccctgacccaccttgaacttgttccacacaggatgccaggccaaggtggagcaagcggtggagacagagccggagcccgagctgcgccagcagaccgagtggcagagcggccagcgctgggaactggcactgggtcgcttttgggattacctgcgctgggtgcagacactgtctgagcaggtgcaggaggagctgctcagctcccaggtcacccaggaactgaggtgagtgtccccatcctggcccttgaccctcctggtgggcggctatacctccccaggtccaggtttcattctgcccctgtcgctaagtcttggggggcctgggtctctgctggttctagcttcctcttcccatttctgactcctggctttagctctctggatatctctctctcagctttgtctctctctcttcccttctgactcagtctctcacactcgtcctggctctgtctctgtccttccctagctcttttatatagagacagagagatggggtctcactgtgttgcccaggctggtcttgaacttctgggctcaagcgatcctcccgcctcggcctcccaaagtgctgggattagaggcatgagccaccttgcccggcctcctagctccttcttcgtctctgcctctgccctctgcatctgctctctgcatctgtctctgtctccttctctcggcctctgccccgttccttctctccctcttgggtctctctggctcatccccatctcgcccgccccatcccagcccttctccccgcctcccactgtgcgacaccctcccgccctctcggccgcagggcgctgatggacgagaccatgaaggagttgaaggcctacaaatcggaactggaggaacaactgaccccggtggcggaggagacgcgggcacggctgtccaaggagctgcaggcggcgcaggcccggctgggcgcggacatggaggacgtgcgcggccgcctggtgcagtaccgcggcgaggtgcaggccatgctcggccagagcaccgaggagctgcgggtgcgcctcgcctcccacctgcgcaagctgcgtaagcggctcctccgcgatgccgatgacctgcagaagcgcctggcagtgtaccaggccggggcccgcgagggcgccgagcgcggcctcagcgccatccgcgagcgcctggggcccctggtggaacagggccgcgtgcgggccgccactgtgggctccctggccggccagccgctacaggagcgggcccaggcctggggcgagcggctgcgcgcgcggatggaggagatgggcagccggacccgcgaccgcctggacgaggtgaaggagcaggtggcggaggtgcgcgccaagctggaggagcaggcccagcagatacgcctgcaggccgaggccttccaggcccgcctcaagagctggttcgagcccctggtggaagacatgcagcgccagtgggccgggctggtggagaaggtgcaggctgccgtgggcaccagcgccgcccctgtgcccagcgacaatcactgaacgccgaagcctgcagccatgcgaccccacgccaccccgtgcctcctgcctccgcgcagcctgcagcgggagaccctgtccccgccccagccgtcctcctggggtggaccctagtttaataaagattcaccaagtttcacgca

SEQ ID NO: 3 - protein, 249 aa, Artificial Sequence
  Mouse Trem2 protein having the R47H point mutation
MGPLHQFLLLLITALSQALNTTVLQGMAGQSLRVSCTYDALKHWGRHKAWCRQLGEEGPCQRVVSTHGVWLLAFLKKRNGSTVIADDTLAGTVTITLKNLQAGDAGLYQCQSLRGREAEVLQKVLVEVLEDPLDDQDAGDLWVPEESSSFEGAQVEHSTSRQVSSCGSPLAYHLPPLSKESRDLLPTHLHSSPPGLRSPEQVSCSQHPLGCGQGQAEAGNTCGQRAGLWPRCWAPTSDPHWTRRYVREF

SEQ ID NO: 4 - DNA, 1056 bp, Artificial Sequence
  DNA encoding mouse Trem2 protein having the R47H point mutation
acttcaagggaaaagcaagatcttgcacaaggtcccctccggctggctgctggcaaaggaaaggtgccatgggacctctccaccagtttctcctgctgctgatcacagccctgtcccaagccctcaacaccacggtgctgcagggcatggccggccagtccttgagggtgtcatgtacttatgacgccttgaagcactgggggagacacaaagcatggtgtcggcagctgggtgaggagggcccatgccagcgtgtggtgagcacacacggtgtgtggctgctggccttcctgaagaagcggaatgggagcacagtcatcgcagatgacacccttgctggaaccgtcaccatcactctgaagaacctccaagccggtgacgcgggcctctaccagtgtcagagtctccgaggccgagaggctgaggtcctgcagaaagtactggtggaggtgctggaggaccctctagatgaccaagatgctggagatctctgggtccccgaggagtcatcgagtttcgagggtgcccaagtggaacacagcacctccaggcaggtttcatcctgtgggtcacctctagcctaccaccttcctcctctttccaaggaatcaagagacctccttcccacccacctccattcttctcctcctggcctgcgttctcctgagcaagtttcttgcagccagcatcctctgggctgtggccaggggcaggcagaagccgggaacacctgtggtcagagggctggactgtggccaagatgctgggcaccaacttcagatcctcactggacccggaggtacgtgagagaattctgagtgggaggagaactacagcttaagtccagccaggagtcaatccagcctgcatgctctcccctcctccaccaagacttctgtttctgctacttttgcttcagaggccgcctctgcctcaagcccacctatcctgggagcaggaatactggtgtgtacatctgtgttgagtggggaagacagctggatggttgtctgtcaacttctgcactttggacattaaacattctccacacaccaa

SEQ ID NO: 5 - protein, 249 aa, Mus musculus
MGPLHQFLLLLITALSQALNTTVLQGMAGQSLRVSCTYDALKHWGRRKAWCRQLGEEGPCQRVVSTHGVWLLAFLKKRNGSTVIADDTLAGTVTITLKNLQAGDAGLYQCQSLRGREAEVLQKVLVEVLEDPLDDQDAGDLWVPEESSSFEGAQVEHSTSRQVSSCGSPLAYHLPPLSKESRDLLPTHLHSSPPGLRSPEQVSCSQHPLGCGQGQAEAGNTCGQRAGLWPRCWAPTSDPHWTRRYVREF

SEQ ID NO: 6 - DNA, 1056 bp, Mus musculus
acttcaagggaaaagcaagatcttgcacaaggtcccctccggctggctgctggcaaaggaaaggtgccatgggacctctccaccagtttctcctgctgctgatcacagccctgtcccaagccctcaacaccacggtgctgcagggcatggccggccagtccttgagggtgtcatgtacttatgacgccttgaagcactgggggagacgcaaggcctggtgtcggcagctgggtgaggagggcccatgccagcgtgtggtgagcacacacggtgtgtggctgctggccttcctgaagaagcggaatgggagcacagtcatcgcagatgacacccttgctggaaccgtcaccatcactctgaagaacctccaagccggtgacgcgggcctctaccagtgtcagagtctccgaggccgagaggctgaggtcctgcagaaagtactggtggaggtgctggaggaccctctagatgaccaagatgctggagatctctgggtccccgaggagtcatcgagtttcgagggtgcccaagtggaacacagcacctccaggcaggtttcatcctgtgggtcacctctagcctaccaccttcctcctctttccaaggaatcaagagacctccttcccacccacctccattcttctcctcctggcctgcgttctcctgagcaagtttcttgcagccagcatcctctgggctgtggccaggggcaggcagaagccgggaacacctgtggtcagagggctggactgtggccaagatgctgggcaccaacttcagatcctcactggacccggaggtacgtgagagaattctgagtgggaggagaactacagcttaagtccagccaggagtcaatccagcctgcatgctctcccctcctccaccaagacttctgtttctgctacttttgcttcagaggccgcctctgcctcaagcccacctatcctgggagcaggaatactggtgtgtacatctgtgttgagtggggaagacagctggatggttgtctgtcaacttctgcactttggacattaaacattctccacacaccaa

SEQ ID NO: 7 - DNA, 20 bp, Artificial Sequence
  Trem2 CRISPR guide
gaagcactgggggagacgca

SEQ ID NO: 8 - DNA, 183 bp, Artificial Sequence
  Trem2 repair oligonucleotide containing a nucleotide G>A point mutation (at nucleotide 89 in this oligo sequence) for  R47H and 2 silent mutations (lysine AAG>AAA (at nucleotide 93) and alanine GCC>GCA (at nucleotide 96)
gccctcaacaccacggtgctgcagggcatggccggccagtccttgagggtgtcatgtacttatgacgccttgaagcactgggggagacacaaagcatggtgtcggcagctgggtgaggagggcccatgccagcgtgtggtgagcacacacggtgtgtggctgctggccttcctgaagaagcgg

SEQ ID NO: 9 - DNA, 4980 bp, Mus musculus
cctgtatctcagggttgagagggaagagagtggggtttccagatgcccacatcccttgatacctagtcctcacccaactctgctctcctagtgaacaactggttggctacagtaacgctgggccaggcaggcatgcatgcgacgtattaccacaaagccagtgaccaggtgagccggagggagcgcctagctgtgggtcccaggctgggtttgctggtgcagttggtatgcccaggagtcctaatgggccactcacatgtgtgccgggccctctctcccccagctgcaggtgggtgtggagtttgaggccagcaccaggatgcaggacaccagtgcctcctttgggtatcagctggacctgcccaaggccaacttcctttttaaaggtaaggaaggcctcagcttccctcctggggaacaggccagataagactcagctgtctgtggtagagtccatgggaaatagggaggttgaacatgtgctggtggagtgggcggggactctgtgcagctccaaattactctgggtggcttgtcaaacagtggggctcctaccctggcatgtttagtacatgttgggggcctcgctttaagccctctcttcccattcccatctagcaagctctctggccctccccactcactcttaccttacttggagttcttctattgtgtgatgaaacactatgatggtaaacagcttagggagcaaagaggttatgttgggttacaactctcaggtggcatgcctaccactgaggagaagatggggcaggactcagcagaaagctgaaggcaagctgatgcagaaggccttgtgggagtgctgcttgttggcttgctccttatggcttcctcagcctgctcttatagcctccggaccattagcccagggtgccccactgaaaataatctgggtactcccacatcaatcacttagaaagtgccctacaggcttgcctgctgccctagctaatggagacatatgtattgaggttccctcagctggatctcttgagttcaagaccagcctggtctacagagcaagttctgggacagccagggctacccagagaaaccctgtctcagaaaagaaaaaaaagaaaaaggtgggggtggggtgactagcttgtataaaactagccagcacagcagggaagctgtgtgaatagtgacagccaggttcagaacctcattctgcgcagtgacatgggtttgtcaagcctgggcggtgttgagccacttaaagggttgctgtgatggtctggagtggccttggttgtgacttaggacatacgggtccgttgtggctaccatagagatgggtggccaggcacatcaagccacccagtctctgccccgctctcggcccacaggctctgtgaacagtaactggatcgtgggcgccacgctggagaagaagcttccgcccttgcccctgacactgtccctctgcgccttcctgaaccaccgcaagaataagttcctgtgtggcttcggcctcaccatcggctgagccctcctgtccttcctctgcagaccatcgctgggccggctgccctcccctcctctccctctctcttggggttggggcagtgggaaggaggggacctcccatgcccaaggatccccagcgccaggggacagtgcccagggggcctggggtcccggagggagtcctgggatctgaagggcattcgattgtgagcgcccaggcagaggcgcagaggcggctgtacacaggctcagaaaggaaagacttgatgtcctcctgagggcagcagaggagcgccgagccgcctgtcacttccccctccacccctccatagaaatcatgtttataagttatggaaaaccgggacattttacagaaaaaaaaaaacttaaaaaacaaaaaatatacgtggaaaaaaaaataggatctgggaggcctcggttttctccagttgttgacatggttgccagcaggcggcgccgagggttcagaaagcacagcagcaccaagcagtttagagaaagcttggccaggcatggtcacaccctctgctcttggggacttacactgccggaacatcagaggcctggcctcaccaggagggtggctccaggtcactcgcctctgtgcagtctggccccgagagctggcagaggactttgtctctgtaaacagggtgggggcagggagacggggctcaggagcctccctgtcccaaaacgggctgaggtggtagcttgtgctgactttctcccagtgggaaggtcagaggtctcagaaacttcaggaagaaacggagttcctggaagttcagcacaataaggaaagttactctgggaggaacgggccctagcaccttcccaggctgaaacaggaaatgtcaagttgttttgttttttaaattttgttgaagatgtagctctgggcctcacgtgtcaggcaggtgctgctgggttccctatagtgcttttccgtgaggcctgctctggggtgtgcgataagggcctcagattgggctctgcatctcactgctgcacctcatggcatcccaagggaagcaaagactcacgatgaactggtcagtgtcctagaccgcagcactaagaccctctctactgcctgggctggagatgggagctggcccttagcaacccatgaaaatcatctcaccacacccagtccttgccagtgttttctgaagccaaagctaacaggcctgggcctggccaggcaccctgtacgtacccttggagccaggtgttccgcctctgcccatcctgcagaatcatgttttgccgtgtctggtgccaaacactgctatgtggcttctctcctgccatcaacagctgggaacagggaaccttgtgcaggcagtgcttctagcaagcttgctgtggtctctgagccccttgtcctacctgacttcccaggtacaatggctttcccactttttgggggttttgttgttgttgggtttttttttgtttttcaagacagggtttctctgtgtagtcctgtcggtcctggaactcactttgtagaccaggctggcctccaactcagaaattcacctgcctctgcctccaagtgctgggattatgggattaaaggcatgtgccaccacgcccagctggcttttccactttttagccaggacttcattctattacctgagctcgggatcttcctgcctcagctttgcatatggctagcactatagacccatgttccagtgaatgacttatggcttgtctttttttttttttttttttttttttatgtgcattagtgttttgcctgcatgtatgccttcgtgagggtagcagatcttggtgttacagttgtgagctgctgtgtgggtgctgcgattttgaacctaggtcctgtgaaatgcagtcagtgctcctaacctctgagtcatctctccagctcctgctcttctgcttttatgaggaaaaagaaaagagaagtggcttgagagtggaaaatgcacatgcaggggtgcacacctgcagtcccagcatgctacagcagaggcagaaggacctttgtgggttagagggcagcctgagaatcttatctcaaaacaactttttaaaatgtgctctgtaggggtagctcttccctcccaaggtgacacatctggcaatcgccagaaacagatcaggagcatcaacgcttggtttcccagggcttggcttaatgtatggcttcaaacccatcgggagccaccactgaacagctcctgaaggaactggagcacgtcccagccttggaatggaaagagttcacctgtggtggaggaatcaacaacgagggatcccagaacaacgatcttcaccccagaagctgagcctcttagcccccacccacccatttccatttaggctgccagctcttttctttacaatgcaccagaccccgcggggaaagggaaggagcggttctcagtgccccagtaccaaggcctggattattcaatgaggtgtccgctccctttgttggcgggggaggggagcggggggtcacaaggcatccaaactccacctctttcctctgccctgctgtgaagggggagagaacaacccgcctcgtgacagggggctggcacagcccgccctagccctgaggagggggcgggacagggggagtcctataattggaccggtctgggatccgatcccctgctcagaccctggaggctaaggacttgtttcggaaggagctggtaagacaagctgggctggggattcacccagggaccttggtaggatgtgggctgggaaccttgagatcccccggagtccaggaaacaggcacaagaattggaaaagcaggcagcacgatagaagtcttgggggacaaactaaggactcgaggtaactagcctttgccagagtcagagcaggtggaggggttacctccaggaaggagtacgggactgtcggtgcacggcgtaccggctcaactaggaaccatcctatggcgaaaaaactcgggatgagccttaggctgcttttatataaatacctactgatttccatcacagtccccaagtaacccggactggtttcaaactgtggctcctcatggctgagctccctaagttctgtagttgtgggagggtaccacttcgcagggatggaggacgattaaaaatcgtgttaaattaacacaaaatggaaagcaggacttagccgggaagaaagaggaatgtaagctggaccacccgctggccctctgtgaagtggaatttgaaccctaggagagggagctggaatttttggcagcggatccaccccggggtgccgagatagcgaactcggcaaggggaggtaaacagacctttgggaagagcgggtgctctgttttggagatgtttgtgatggctcacagatctgagaagggaagatggggttctctgggtggccggagtccctccacccccgccccctggtgttcaaagacaatttttccctccgcag

SEQ ID NO: 10 - DNA, 4292 bp, Homo sapiens
actggccaatcacaggcaggaagatgaaggttctgtgggctgcgttgctggtcacattcctggcaggtatgggggcggggcttgctcggttccccccgctcctccccctctcatcctcacctcaacctcctggccccattcaggcagaccctgggccccctcttctgaggcttctgtgctgcttcctggctctgaacagcgatttgacgctctctgggcctcggtttcccccatccttgagataggagttagaagttgttttgttgttgttgtttgttgttgttgttttgtttttttgagatgaagtctcgctctgtcgcccaggctggagtgcagtggcgggatctcggctcactgcaagctccgcctcccaggtccacgccattctcctgcctcagcctcccaagtagctgggactacaggcacatgccaccacacccgactaacttttttgtattttcagtagagacggggtttcaccatgttggccaggctggtctggaactcctgacctcaggtgatctgcccgtttcgatctcccaaagtgctgggattacaggcgtgagccaccgcacctggctgggagttagaggtttctaatgcattgcaggcagatagtgaataccagacacggggcagctgtgatctttattctccatcacccccacacagccctgcctggggcacacaaggacactcaatacatgcttttccgctgggcgcggtggctcacccctgtaatcccagcactttgggaggccaaggtgggaggatcacttgagcccaggagttcaacaccagcctgggcaacatagtgagaccctgtctctactaaaaatacaaaaattagccaggcatggtgccacacacctgtgctctcagctactcaggaggctgaggcaggaggatcgcttgagcccagaaggtcaaggttgcagtgaaccatgttcaggccgctgcactccagcctgggtgacagagcaagaccctgtttataaatacataatgctttccaagtgattaaaccgactcccccctcaccctgcccaccatggctccaaagaagcatttgtggagcaccttctgtgtgcccctaggtactagatgcctggacggggtcagaaggaccctgacccaccttgaacttgttccacacaggatgccaggccaaggtggagcaagcggtggagacagagccggagcccgagctgcgccagcagaccgagtggcagagcggccagcgctgggaactggcactgggtcgcttttgggattacctgcgctgggtgcagacactgtctgagcaggtgcaggaggagctgctcagctcccaggtcacccaggaactgaggtgagtgtccccatcctggcccttgaccctcctggtgggcggctatacctccccaggtccaggtttcattctgcccctgtcgctaagtcttggggggcctgggtctctgctggttctagcttcctcttcccatttctgactcctggctttagctctctggatatctctctctcagctttgtctctctctcttcccttctgactcagtctctcacactcgtcctggctctgtctctgtccttccctagctcttttatatagagacagagagatggggtctcactgtgttgcccaggctggtcttgaacttctgggctcaagcgatcctcccgcctcggcctcccaaagtgctgggattagaggcatgagccaccttgcccggcctcctagctccttcttcgtctctgcctctgccctctgcatctgctctctgcatctgtctctgtctccttctctcggcctctgccccgttccttctctccctcttgggtctctctggctcatccccatctcgcccgccccatcccagcccttctccccgcctcccactgtgcgacaccctcccgccctctcggccgcagggcgctgatggacgagaccatgaaggagttgaaggcctacaaatcggaactggaggaacaactgaccccggtggcggaggagacgcgggcacggctgtccaaggagctgcaggcggcgcaggcccggctgggcgcggacatggaggacgtgcgcggccgcctggtgcagtaccgcggcgaggtgcaggccatgctcggccagagcaccgaggagctgcgggtgcgcctcgcctcccacctgcgcaagctgcgtaagcggctcctccgcgatgccgatgacctgcagaagcgcctggcagtgtaccaggccggggcccgcgagggcgccgagcgcggcctcagcgccatccgcgagcgcctggggcccctggtggaacagggccgcgtgcgggccgccactgtgggctccctggccggccagccgctacaggagcgggcccaggcctggggcgagcggctgcgcgcgcggatggaggagatgggcagccggacccgcgaccgcctggacgaggtgaaggagcaggtggcggaggtgcgcgccaagctggaggagcaggcccagcagatacgcctgcaggccgaggccttccaggcccgcctcaagagctggttcgagcccctggtggaagacatgcagcgccagtgggccgggctggtggagaaggtgcaggctgccgtgggcaccagcgccgcccctgtgcccagcgacaatcactgaacgccgaagcctgcagccatgcgaccccacgccaccccgtgcctcctgcctccgcgcagcctgcagcgggagaccctgtccccgccccagccgtcctcctggggtggaccctagtttaataaagattcaccaagtttcacgcatctgctggcctccccctgtgatttcctctaagccccagcctcagtttctctttctgcccacatactggccacacaattctcagccccctcctctccatctgtgtctgtgtgtatctttctctctgcccttttttttttttttagacggagtctggctctgtcacccaggctagagtgcagtggcacgatcttggctcactgcaacctctgcctcttgggttcaagcgattctgctgcctcagtagctgggattacaggctcacaccaccacacccggctaatttttgtatttttagtagagacgagctttcaccatgttggccaggcaggtctcaaactcctgaccaagtgatccacccgccggcctcccaaagtgctgagattacaggcctgagccaccatgcccggcctctgcccctctttcttttttagggggcagggaaaggtctcaccctgtcacccgccatcacagctcactgcagcctccacctcctggactcaagtgataagtgatcctcccgcctcagcctttccagtagctgagactacaggcgcataccactaggattaatttgggggggggggtggtgtgtgtggagatggggtctggctttgttggccaggctgatgtggaattcctgggctcaagcgatactcccaccttggcctcctgagtagctgagactactggctagcaccaccacacccagctttttattattatttgtagagacaaggtctcaatatgttgcccaggctagtctcaaacccctgggctcaagagatcctccgccatcggcctcccaaagtgctgggattccaggcatggggctccgagcccggcctgcccaacttaataatacttgttcctcagagttgcaactccaaatgacctgagattggtgcctttattctaagctattttcattttttttctgctgtcattattctcccccttctctcctccagtcttatctgatatctgcctccttcccacccaccctgcaccccatcccacccctctgtctctccctgttctcctcaggagactctggcttcctgttttcctccacttctatcttttatctctccctcctacggtttcttttctttctccccggcctgcttgtttctcccccaacccccttcatctggatttcttcttctgccattcagtttggtttgagctctctgcttctccggttccctctgagctagctgtcccttcacccactgtgaactgggtttccctgcccaaccctcattctctttctttctttctttttttttttttttttttttttttttttttgagacagagtcttgctctgttgcccagcctggagtgcagtggtgcaatcttggttcactgcaacctccacttcccagattcaagcaattctcctgcctcagcctccagagtagctgggattacaggcgtgtcccaccacacccgactaatttttgtatttttggtagagacaaggcttcggcattgtt

SEQ ID NO: 11 - DNA, 1834 bp, Artificial Sequence
  A Frt PGKneo Frt cassette followed by an Nde1 restriction enzyme site (CATATG)
gaagttcctattctctagaaagtataggaacttcaggtctgaagaggagtttacgtccagccaagctagcttggctgcaggtcgtcgaaattctaccgggtaggggaggcgcttttcccaaggcagtctggagcatgcgctttagcagccccgctgggcacttggcgctacacaagtggcctctggcctcgcacacattccacatccaccggtaggcgccaaccggctccgttctttggtggccccttcgcgccaccttctactcctcccctagtcaggaagttcccccccgccccgcagctcgcgtcgtgcaggacgtgacaaatggaagtagcacgtctcactagtctcgtgcagatggacagcaccgctgagcaatggaagcgggtaggcctttggggcagcggccaatagcagctttgctccttcgctttctgggctcagaggctgggaaggggtgggtccgggggcgggctcaggggcgggctcaggggcggggcgggcgcccgaaggtcctccggaggcccggcattctgcacgcttcaaaagcgcacgtctgccgcgctgttctcctcttcctcatctccgggcctttcgacctgcagcctgttgacaattaatcatcggcatagtatatcggcatagtataatacgacaaggtgaggaactaaaccatgggatcggccattgaacaagatggattgcacgcaggttctccggccgcttgggtggagaggctattcggctatgactgggcacaacagacaatcggctgctctgatgccgccgtgttccggctgtcagcgcaggggcgcccggttctttttgtcaagaccgacctgtccggtgccctgaatgaactgcaggacgaggcagcgcggctatcgtggctggccacgacgggcgttccttgcgcagctgtgctcgacgttgtcactgaagcgggaagggactggctgctattgggcgaagtgccggggcaggatctcctgtcatctcaccttgctcctgccgagaaagtatccatcatggctgatgcaatgcggcggctgcatacgcttgatccggctacctgcccattcgaccaccaagcgaaacatcgcatcgagcgagcacgtactcggatggaagccggtcttgtcgatcaggatgatctggacgaagagcatcaggggctcgcgccagccgaactgttcgccaggctcaaggcgcgcatgcccgacggcgatgatctcgtcgtgacccatggcgatgcctgcttgccgaatatcatggtggaaaatggccgcttttctggattcatcgactgtggccggctgggtgtggcggaccgctatcaggacatagcgttggctacccgtgatattgctgaagagcttggcggcgaatgggctgaccgcttcctcgtgctttacggtatcgccgctcccgattcgcagcgcatcgccttctatcgccttcttgacgagttcttctgaggggatcaattctctagagctcgctgatcagcctcgactgtgccttctagttgccagccatctgttgtttgcccctcccccgtgccttccttgaccctggaaggtgccactcccactgtcctttcctaataaaatgaggaaattgcatcgcattgtctgagtaggtgtcattctattctggggggtggggtggggcaggacagcaagggggaggattgggaagacaatagcaggcatgctggggatgcggtgggctctatggcttctgaggcggaaagaaccagctggggctcgactagagcttgcggaacccttcgaagttcctattctctagaaagtataggaacttccatatg

SEQ ID NO: 12 - DNA, 5166 bp, Mus musculus
aaacctgatggagaagatacaggcctctgtggctaccaaccccatcatcaccccagtggcccaggagaatcaatgagtatccttctcctgtcctgcaacaacatccatatccagccaggtggccctgtctcaagcacctctctggccctctggtggcccttgcttaataaagattctccgagcacattctgagtctctgtgagtgattccaatcagcttcagcctcagtttattgttttttgccttacctagcacacattccatggccctgtcactatctgtagagggaggtggttttgcagcaatagaaatgaagcctaggacctagcaacataaaagaacaagtgatctaccactgagccacgcccacagcccctcactgggggattctaggcaggggctctaccactgagccacccgcagcccctcactggggaatcatatctaccactgagtcacgcccctccagcccctcactacgggaattctagtcagtagctctaccactgagccacacccacagcctctggggctcttcaccgccccctacccctggattctaggcatgggctcattttatttatttatttatttaagatttgtttatcttatgtataaggtacactgcagctgtcttcaggcgtcaggtcccattacagatggttgtgagccaccatgtggttgctgggaattgaactcaggacttatagaagagtagtcagtgctcttaactgctgagccatctctccagcacccagtacaggctcttctatttagctatatccacccttctttttagtctgaaataggatctcaactgattttccttgcactccctctagcctagtttggtcttgaatatttgaatctttgttttcaaatcaatctctacaggaactgagaaaggcatgtaccacttcatgtgggtcagttgggctacttttcccaacttcccaagcacccactgcacagctatgccttgaatcaatcaacatgtaagagaccagggtcgccaggcggtgtttacttttctggttgtcttatctctcctcctccgctctagtcttatctgacaccctctccttgccttgtctctcctctttttcccttctaggcttccttttctggcttcctgttttcctgatcctctgttatctcaccctcccgcggtttcttttgctctgggcctttggttggcggtttctacggtttctacgtggcttttggaacctcagcctttctcccttgctctgaagttagctggatctttgctccctctgggtcatggggccttagccccattctttctcccctgcctgtgctgcatgccttttgactttcccagcaagtgtatggagagtgagttcaggctggggacacaaaaccattctccccatgtcctggtactcaaaggggtcatggtggaagctggagagcccctggctggcttctcctcccaccccctcagttctcagggactcagcagggctcccactaacaggggcaggctagggcttgagctgtgtcttgggtcgggccaaggcttcagaactcaactgcctctggcacaccccgagcctgcagcttttcctggcatcaaactcagcattatctggaggcaggcaccactcccacacatgactcattaggcccaatgagaagatgggtcggtgggctagtgacagggccctagacagccacacttcatgcccaggggctaggagcacacccccagagcctcactactctcaaatatcaagatgaggggagagtatagagggaatgtctccctctgaagacctgaattattgtgatgttatttgagccacgctggccttgaactctgaaccctcctgcctcatcttcaaaggctggaattacaggttcgcgccactaggcctatctgagaacttagttaattctacagaagagagtttgttttcactggtttgaaacgaggcctcgtgtacccagagctactcttttgccaactcactgtagagccaaggatgaccttgaactctggtcttcctggctccgagtcctcggtactgggtagacaatgtgtgatcctaacccccagttttatgtggtgctatacagatggcatccagggtttcctgcatgctggacaggtcatcaaccaaccgagccacatcctcctcatcatcatcactttgttgttggttttcaatccagagctcatggagcccaagctggcctcaatctatataaccaagactgtgcctggtcttcctgtctctacctaacaaatgatggtgggatgcagggatgtacaaccaggagcagagccttacttctaaacgaagaaggaaccccacctccctgtgggcagacctggaggtggggcaaggaccacagaaagacattacagaactaggatcgtgaaggaagtcatggaggccagcctgttgtacagagtgagttccaggacagccagggctacacagaggaaaacaagaaggaaaaaaaaaaaaaaaaaaagaactgaatgactagcagttttagaaccttagctgtgtgcttcccgtaccctacctgtggcacaggaagcccttgttgctaagagtaggatgacactggaagcaccaagcactgggcagagtaagggggaaatctgttacattattcagatgggcgcttgaggactgagcaggactcctttcaagaagcaaaagggtcaggcctggtgcccacagggactggaagctagctagcgccgagttggccccagagatgtcgcaacccagccagggtcgagaatctgttccacccctttcacaaccatccccctgttgtcgtcgtccccacccccacccccgccccaactgacacgtgggttgcaggggcaccaggccagccaacctagagtctgggccccttagccaccagctgccagggggtcactgtcggtcaatgacagctctgggggagggggggagaagggccttggactctagcctgagagaaaggatgttgtggaaggagggggcagggaggcaagtttagggcctgcaggggcctaggaggccccacaagacctaaaaacgggggaaggggggttgtgccagttaggggacactatggagctctgcaagctaagaggctcttagcttctttgcagttttgactagctgaagaggcaacttctaaggaagggagatgaggggatgccaagatcccagagagcatccgaggaggtctgagggtgtgcagatgcaaaggcattggaggtgaagggagccagggtgcagcatccgggacagaatgtgagctgaggctcctggtcaaggagaaggtagagaagagctaacctgaggatgcagtgtgagctaggggtgagatgggggtgaggggagttgtttgtaagacccccccccttaaggtgggacagcctcagagagagagtgagtaggcagagcagccaaggctgggtggagatcaatgagatttggaagtgaggatgctgaccagtgacgagccttgggcctaaataaaaagcctggatgtgggatctgcctcccagtatcgaccagaatgacagaagagagtgggctggttgtgttggtgttggtgcatgcctgtaatcccagcaactcactagagaggcagaggcaggagcatcacaaattccaggccagccaaaaagcctatgtaaaaaaaaaaaaaagagaaaaaagaaaaaagaaaaagtaggtggacacagagacaagggggaggctcagggggagggcgaccagcttgctccgccccctccccaaccggttaaacctctgtgcaggatcctcccaccgccatgggcctcctgagagatccttagatccaggttagtgcataggaaagtgtccccccactacctacagctaagggattggggtggtgggatcatggtggagggcggtggtgaatactagcgatgtcccccgctacccgtgcgtctgcctccagggtgcccctccaaccaggatgaggctcttcatcgctcttcctgtcctgattgtggtcgtagccatgaccttggaaggtaagaaagagccttggaaggtaagaaagaggcttggaagtgtgaagttggccttgtgcctgcggcccaggcttagaagaccctcgaggagggctctgaggtccctttctgtgtcatcattccactaccgccctcccatcgtcccccatcccacctgccaggtgccttatttttgtgtcaaagtgggtgctgaaggaggcaactctgtccagaaaagacgcagtaaccaatgacctaggataccaccctttggaattggctaatcttcctagaaggggcggagcgtaaaaacaaggaggtgagaggtgcagtaaaatcaagtgtccaataccctcccccatgctaatgagtttgctcgcaaccctctcgcggcaggcccagcccccgcccaggcggccccggatttgtccggaacattggagagcataccggataaactgaaggagtttgggaacactttggaagacaaggcccgggcagccattgaacatatcaaacagaaggaaattttgaccaagacccggttaggacctttcagggcacgggcgggtggtgtgtgtgtgtgtgcgtgcgcgcgcgcccgtgtgtaaaagccctagcagacagttccacactgacacaatggggaaactgcaccagagtgtttgacactttccctgaagtcatagaactgtatctgaagtcattgaactggatgtcaaagtgctcgtagtgtggagacaggcggtgtaactcccagccaactgttagagatgtttccaagtcctagtgaagggccaagctaggcggctgactggttaggacagaccctgacccctccctgtgtactcttgagacaggtcatgacttgagtctccgagacagagaaagaatgtaggagagttggggcaggggcacagcagaagctgtacaggcctgggctctgcagtttacactggccaaagagagattagggcatgctgggttaagaactagccaggcagtggtggcgcacacctttgatcccagtattcatgaggcagaggcaggcagatctctttgaggccagcctgattggagctagttctaggaaagccagggctacacagagaaaccctgtctcaacaccaccaccacccccc

SEQ ID NO: 13 - protein, 311 aa, Mus musculus
MKALWAVLLVTLLTGCLAEGEPEVTDQLEWQSNQPWEQALNRFWDYLRWVQTLSDQVQEELQSSQVTQELTALMEDTMTEVKAYKKELEEQLGPVAEETRARLGKEVQAAQARLGADMEDLRNRLGQYRNEVHTMLGQSTEEIRARLSTHLRKMRKRLMRDAEDLQKRLAVYKAGAREGAERGVSAIRERLGPLVEQGRQRTANLGAGAAQPLRDRAQAFGDRIRGRLEEVGNQARDRLEEVREHMEEVRSKMEEQTQQIRLQAEIFQARLKGWFEPIVEDMHRQWANLMEKIQASVATNPIITPVAQENQ

SEQ ID NO: 14 - protein, 317 aa, Homo sapiens [sequence omitted]

SEQ ID NO: 15 - protein, 299 aa, Homo sapiens
KVEQAVETEPEPELRQQTEWQSGQRWELALGRFWDYLRWVQTLSEQVQEELLSSQVTQELRALMDETMKELKAYKSELEEQLTPVAEETRARLSKELQAAQARLGADMEDVRGRLVQYRGEVQAMLGQSTEELRVRLASHLRKLRKRLLRDADDLQKRLAVYQAGAREGAERGLSAIRERLGPLVEQGRVRAATVGSLAGQPLQERAQAWGERLRARMEEMGSRTRDRLDEVKEQVAEVRAKLEEQAQQIRLQAEAFQARLKSWFEPLVEDMQRQWAGLVEKVQAAVGTSAAPVPSDNH

SEQ ID NO: 16 - protein, 7 aa, Simian virus 40
PKKKRKV

SEQ ID NO: 17 - protein, 14 aa, Xenopus laevis
RPAATKKAGQAKKK